European Patent Specification EP 3 980 047 B1, published February 14, 2024. Title: INFLAMMATORY DISEASE TREATMENT WITH COMPLEMENT INHIBITORS. Applicant: RA PHARMACEUTICALS, INC. Application PCT/US2020/XXXXXX. The sequence listing filed with the application follows.

SEQUENCE LISTING (1 sequence)

SEQ ID NO: 1 - protein, 15 aa, Artificial Sequence
  source: /note="Description of Artificial Sequence: Synthetic peptide"
  source: /note="N-term Ac"
  SITE (1)..(6): /note="Lactam bridge between residues"
  MOD_RES (7)..(7): N-methyl-aspartic acid
  MOD_RES (8)..(8): Tert-butylglycine
  MOD_RES (10)..(10): 7-azatryptophan
  MOD_RES (14)..(14): Cyclohexylglycine
  MOD_RES (15)..(15): N-epsilon-(PEG24-gamma-glutamic acid-N-alpha-hexadecanoyl)Lys
KVERFDXXYXEYPXK